European Patent Application EP 4 293 046 A1, published December 20, 2023. Title: ANTI-PD-1 ANTIBODY AND USE THEREOF. Applicant: SHANGHAI JEMINCARE PHARMACEUTICAL CO., LTD.; JIANGXI JEMINCARE GROUP CO., LTD. The sequence listing filed with the application follows.

SEQUENCE LISTING (87 sequences)

SEQ ID NO: 1 - protein, 7 aa, Artificial Sequence
  41D2-2C3D7 HCDR1
GFTFSNY

SEQ ID NO: 2 - protein, 6 aa, Artificial Sequence
  41D2-2C3D7 HCDR2
SGGGSY

SEQ ID NO: 3 - protein, 7 aa, Artificial Sequence
  41D2-2C3D7 HCDR3
PYYGMEY

SEQ ID NO: 4 - protein, 25 aa, Artificial Sequence
  41D2-2C3D7 H-FR1
EVKLVESGGGLVKPGGSLKLACAAS

SEQ ID NO: 5 - protein, 19 aa, Artificial Sequence
  41D2-2C3D7 H-FR2
DMSWVRQTPEKRLEWVATI

SEQ ID NO: 6 - protein, 41 aa, Artificial Sequence
  41D2-2C3D7 H-FR3
TYYPDSVKGRFTISRDNAKNNLYLQMSSLRSEDTALYYCVS

SEQ ID NO: 7 - protein, 11 aa, Artificial Sequence
  41D2-2C3D7 H-FR4
WGQGTSVTVSS

SEQ ID NO: 8 - protein, 11 aa, Artificial Sequence
  41D2-2C3D7 LCDR1
KASQDVGTAVA

SEQ ID NO: 9 - protein, 7 aa, Artificial Sequence
  41D2-2C3D7 LCDR2
WASTRHT

SEQ ID NO: 10 - protein, 9 aa, Artificial Sequence
  41D2-2C3D7 LCDR3
QQYSSYPWT

SEQ ID NO: 11 - protein, 23 aa, Artificial Sequence
  41D2-2C3D7 L-FR1
DIVMTQSHKFMSTSVGDRVSITC

SEQ ID NO: 12 - protein, 15 aa, Artificial Sequence
  41D2-2C3D7 L-FR2
WYQQKPGQSPKLLIY

SEQ ID NO: 13 - protein, 32 aa, Artificial Sequence
  41D2-2C3D7 L-FR3
GVPDRFTGSGSGTDFTLTISNVQSEDLADYFC

SEQ ID NO: 14 - protein, 10 aa, Artificial Sequence
  41D2-2C3D7 L-FR4
FGGGTKLEVK

SEQ ID NO: 15 - protein, 116 aa, Artificial Sequence
  41D2-2C3D7 VH
EVKLVESGGGLVKPGGSLKLACAASGFTFSNYDMSWVRQTPEKRLEWVATISGGGSYTYYPDSVKGRFTISRDNAKNNLYLQMSSLRSEDTALYYCVSPYYGMEYWGQGTSVTVSS

SEQ ID NO: 16 - protein, 107 aa, Artificial Sequence
  41D2-2C3D7 VL
DIVMTQSHKFMSTSVGDRVSITCKASQDVGTAVAWYQQKPGQSPKLLIYWASTRHTGVPDRFTGSGSGTDFTLTISNVQSEDLADYFCQQYSSYPWTFGGGTKLEVK

SEQ ID NO: 17 - protein, 25 aa, Artificial Sequence
  1910D2HzH3 H-FR1
EVQLVESGGGLVKPGGSLRLSCAAS

SEQ ID NO: 18 - protein, 19 aa, Artificial Sequence
  1910D2HzH3 H-FR2
DMSWVRQAPGKGLEWVSTI

SEQ ID NO: 19 - protein, 41 aa, Artificial Sequence
  1910D2HzH3 H-FR3
TYYADSVKGRFTISRDNAKNSLYLQMNSLRAEDTAVYYCVS

SEQ ID NO: 20 - protein, 11 aa, Artificial Sequence
  1910D2HzH3 H-FR4
WGQGTLVTVSS

SEQ ID NO: 21 - protein, 23 aa, Artificial Sequence
  1910D2HzL4 L-FR1
DIQLTQSPSFLSASVGDRVTITC

SEQ ID NO: 22 - protein, 15 aa, Artificial Sequence
  1910D2HzL4 L-FR2
WYQQKPGKAPKLLIY

SEQ ID NO: 23 - protein, 32 aa, Artificial Sequence
  1910D2HzL4 L-FR3
GVPSRFSGSGSGTEFTLTISSLQPEDFATYFC

SEQ ID NO: 24 - protein, 10 aa, Artificial Sequence
  1910D2HzL4 L-FR4
FGGGTKVEIK

SEQ ID NO: 25 - protein, 116 aa, Artificial Sequence
  1910D2HzH3 VH
EVQLVESGGGLVKPGGSLRLSCAASGFTFSNYDMSWVRQAPGKGLEWVSTISGGGSYTYYADSVKGRFTISRDNAKNSLYLQMNSLRAEDTAVYYCVSPYYGMEYWGQGTLVTVSS

SEQ ID NO: 26 - protein, 107 aa, Artificial Sequence
  1910D2HzL4 VL
DIQLTQSPSFLSASVGDRVTITCKASQDVGTAVAWYQQKPGKAPKLLIYWASTRHTGVPSRFSGSGSGTEFTLTISSLQPEDFATYFCQQYSSYPWTFGGGTKVEIK

SEQ ID NO: 27 - protein, 5 aa, Artificial Sequence
  46H3A8 HCDR1
DYEMH

SEQ ID NO: 28 - protein, 17 aa, Artificial Sequence
  46H3A8 HCDR2
GIHPGSGGTAYNQKFKG

SEQ ID NO: 29 - protein, 11 aa, Artificial Sequence
  46H3A8 HCDR3
EGFDVGWYFDV

SEQ ID NO: 30 - protein, 30 aa, Artificial Sequence
  46H3A8 H-FR1
QVQLQQSGAELVRPGASVKLSCKALGFTFI

SEQ ID NO: 31 - protein, 14 aa, Artificial Sequence
  46H3A8 H-FR2
WVRQTPVHGLEWIG

SEQ ID NO: 32 - protein, 32 aa, Artificial Sequence
  46H3A8 H-FR3
KATLIADISTNTASMEVSSLTSEDSAVYYCTR

SEQ ID NO: 33 - protein, 11 aa, Artificial Sequence
  46H3A8 H-FR4
WGAGTTVTVSS

SEQ ID NO: 34 - protein, 16 aa, Artificial Sequence
  46H3A8 LCDR1
RSSQSIVHSDGDTFLE

SEQ ID NO: 35 - protein, 7 aa, Artificial Sequence
  46H3A8 LCDR2
KVSNRFS

SEQ ID NO: 36 - protein, 9 aa, Artificial Sequence
  46H3A8 LCDR3
FQGSHVPYT

SEQ ID NO: 37 - protein, 23 aa, Artificial Sequence
  46H3A8 L-FR1
DVLMTQTPLSLPVSLGDQASISC

SEQ ID NO: 38 - protein, 15 aa, Artificial Sequence
  46H3A8 L-FR2
WYLQKPGQSPKLLIY

SEQ ID NO: 39 - protein, 32 aa, Artificial Sequence
  46H3A8 L-FR3
GVPDRFSGSGSGTDFTLKISRVEGEDLGVYYC

SEQ ID NO: 40 - protein, 10 aa, Artificial Sequence
  46H3A8 L-FR4
FGGGTKLEIK

SEQ ID NO: 41 - protein, 120 aa, Artificial Sequence
  46H3A8 VH
QVQLQQSGAELVRPGASVKLSCKALGFTFIDYEMHWVRQTPVHGLEWIGGIHPGSGGTAYNQKFKGKATLIADISTNTASMEVSSLTSEDSAVYYCTREGFDVGWYFDVWGAGTTVTVSS

SEQ ID NO: 42 - protein, 112 aa, Artificial Sequence
  46H3A8 VL
DVLMTQTPLSLPVSLGDQASISCRSSQSIVHSDGDTFLEWYLQKPGQSPKLLIYKVSNRFSGVPDRFSGSGSGTDFTLKISRVEGEDLGVYYCFQGSHVPYTFGGGTKLEIK

SEQ ID NO: 43 - protein, 30 aa, Artificial Sequence
  1910h3hzH4 H-FR1
QVQLVQSGAEVKKPGASVKVSCKASGFTFI

SEQ ID NO: 44 - protein, 14 aa, Artificial Sequence
  1910h3hzH4 H-FR2
WVRQAPGQGLEWIG

SEQ ID NO: 45 - protein, 32 aa, Artificial Sequence
  1910h3hzH4 H-FR3
RATLTADISISTAYMELSRLRSDDTAVYYCTR

SEQ ID NO: 46 - protein, 11 aa, Artificial Sequence
  1910h3hzH4 H-FR4
WGQGTTVTVSS

SEQ ID NO: 47 - protein, 23 aa, Artificial Sequence
  1910h3hzL3 L-FR1
DVVMTQSPLSLPVTLGQPASISC

SEQ ID NO: 48 - protein, 15 aa, Artificial Sequence
  1910h3hzL3 L-FR2
WYQQRPGQSPRLLIY

SEQ ID NO: 49 - protein, 32 aa, Artificial Sequence
  1910h3hzL3 L-FR3
GVPDRFSGSGSGTDFTLKISRVEAEDVGVYYC

SEQ ID NO: 50 - protein, 10 aa, Artificial Sequence
  1910h3hzL3 L-FR4
FGQGTKLEIK

SEQ ID NO: 51 - protein, 120 aa, Artificial Sequence
  1910h3hzH4 VH
QVQLVQSGAEVKKPGASVKVSCKASGFTFIDYEMHWVRQAPGQGLEWIGGIHPGSGGTAYNQKFKGRATLTADISISTAYMELSRLRSDDTAVYYCTREGFDVGWYFDVWGQGTTVTVSS

SEQ ID NO: 52 - protein, 112 aa, Artificial Sequence
  1910h3hzL3 VL
DVVMTQSPLSLPVTLGQPASISCRSSQSIVHSDGDTFLEWYQQRPGQSPRLLIYKVSNRFSGVPDRFSGSGSGTDFTLKISRVEAEDVGVYYCFQGSHVPYTFGQGTKLEIK

SEQ ID NO: 53 - protein, 95 aa, Homo sapiens
DIQLTQSPSFLSASVGDRVTITCRASQGISSYLAWYQQKPGKAPKLLIYAASTLQSGVPSRFSGSGSGTEFTLTISSLQPEDFATYYCQQLNSYP

SEQ ID NO: 54 - protein, 12 aa, Homo sapiens
LTFGGGTKVEIK

SEQ ID NO: 55 - protein, 98 aa, Homo sapiens
EVQLVESGGGLVKPGGSLRLSCAASGFTFSSYSMNWVRQAPGKGLEWVSSISSSSSYIYYADSVKGRFTISRDNAKNSLYLQMNSLRAEDTAVYYCAR

SEQ ID NO: 56 - protein, 16 aa, Homo sapiens
NWFDSWGQGTLVTVSS

SEQ ID NO: 57 - protein, 25 aa, Artificial Sequence
  41D2-2C3D7 H-FR1; 1910D2HzH3 H-FR1
  misc_feature (3)..(3): Xaa = Lys or Gln
  misc_feature (19)..(19): Xaa = Lys or Arg
  misc_feature (21)..(21): Xaa = Ala or Ser
EVXLVESGGGLVKPGGSLXLXCAAS

SEQ ID NO: 58 - protein, 30 aa, Artificial Sequence
  46H3A8 H-FR1; 1910h3hzH4 H-FR1
  misc_feature (5)..(5): Xaa = Gln or Val
  misc_feature (11)..(11): Xaa = Leu or Val
  misc_feature (12)..(12): Xaa = Lys or Val
  misc_feature (13)..(13): Xaa = Lys or Arg
  misc_feature (20)..(20): Xaa = Leu or Val
  misc_feature (25)..(25): Xaa = Leu or Ser
QVQLXQSGAEXXXPGASVKXSCKAXGFTFI

SEQ ID NO: 59 - protein, 19 aa, Artificial Sequence
  41D2-2C3D7 H-FR2; 1910D2HzH3 H-FR2
  misc_feature (8)..(8): Xaa = Ala or Thr
  misc_feature (10)..(10): Xaa = Glu or Gly
  misc_feature (12)..(12): Xaa = Gly or Arg
  misc_feature (17)..(17): Xaa = Ala or Ser
DMSWVRQXPXKXLEWVXTI

SEQ ID NO: 60 - protein, 14 aa, Artificial Sequence
  46H3A8 H-FR2; 1910h3hzH4 H-FR2
  misc_feature (5)..(5): Xaa = Ala or Thr
  misc_feature (7)..(7): Xaa = Gly or Val
  misc_feature (8)..(8): Xaa = His or Gln
WVRQXPXXGLEWIG

SEQ ID NO: 61 - protein, 41 aa, Artificial Sequence
  41D2-2C3D7 H-FR3; 1910D2HzH3 H-FR3
  misc_feature (4)..(4): Xaa = Ala or Pro
  misc_feature (21)..(21): Xaa = Asn or Ser
  misc_feature (27)..(27): Xaa = Asn or Ser
  misc_feature (31)..(31): Xaa = Ala or Ser
  misc_feature (36)..(36): Xaa = Leu or Val
TYYXDSVKGRFTISRDNAKNXLYLQMXSLRXEDTAXYYCVS

SEQ ID NO: 62 - protein, 32 aa, Artificial Sequence
  46H3A8 H-FR3; 1910h3hzH4 H-FR3
  misc_feature (1)..(1): Xaa = Lys or Arg
  misc_feature (5)..(5): Xaa = Ile or Thr
  misc_feature (10)..(10): Xaa = Ile or Thr
  misc_feature (11)..(11): Xaa = Asn or Ser
  misc_feature (14)..(14): Xaa = Ser or Tyr
  misc_feature (17)..(17): Xaa = Leu or Val
  misc_feature (19)..(19): Xaa = Arg or Ser
  misc_feature (21)..(21): Xaa = Arg or Thr
  misc_feature (23)..(23): Xaa = Asp or Glu
  misc_feature (25)..(25): Xaa = Ser or Thr
XATLXADISXXTAXMEXSXLXSXDXAVYYCTR

SEQ ID NO: 63 - protein, 11 aa, Artificial Sequence
  41D2-2C3D7 H-FR4; 1910D2HzH3 H-FR4
  misc_feature (6)..(6): Xaa = Leu or Ser
WGQGTXVTVSS

SEQ ID NO: 64 - protein, 11 aa, Artificial Sequence
  46H3A8 H-FR4; 1910h3hzH4 H-FR4
  misc_feature (3)..(3): Xaa = Ala or Gln
WGXGTTVTVSS

SEQ ID NO: 65 - protein, 116 aa, Artificial Sequence
  41D2-2C3D7 VH; 1910D2HzH3 VH
  misc_feature (3)..(3): Xaa = Lys or Gln
  misc_feature (19)..(19): Xaa = Lys or Arg
  misc_feature (21)..(21): Xaa = Ala or Ser
  misc_feature (40)..(40): Xaa = Ala or Thr
  misc_feature (42)..(42): Xaa = Glu or Gly
  misc_feature (44)..(44): Xaa = Gly or Arg
  misc_feature (49)..(49): Xaa = Ala or Ser
  misc_feature (61)..(61): Xaa = Ala or Pro
  misc_feature (78)..(78): Xaa = Asn or Ser
  misc_feature (84)..(84): Xaa = Asn or Ser
  misc_feature (88)..(88): Xaa = Ala or Ser
  misc_feature (93)..(93): Xaa = Leu or Val
  misc_feature (111)..(111): Xaa = Leu or Ser
EVXLVESGGGLVKPGGSLXLXCAASGFTFSNYDMSWVRQXPXKXLEWVXTISGGGSYTYYXDSVKGRFTISRDNAKNXLYLQMXSLRXEDTAXYYCVSPYYGMEYWGQGTXVTVSS

SEQ ID NO: 66 - protein, 120 aa, Artificial Sequence
  46H3A8 VH; 1910h3hzH4 VH
  misc_feature (5)..(5): Xaa = Gln or Val
  misc_feature (11)..(11): Xaa = Leu or Val
  misc_feature (12)..(12): Xaa = Lys or Val
  misc_feature (13)..(13): Xaa = Lys or Arg
  misc_feature (20)..(20): Xaa = Leu or Val
  misc_feature (25)..(25): Xaa = Leu or Ser
  misc_feature (40)..(40): Xaa = Ala or Thr
  misc_feature (42)..(42): Xaa = Gly or Val
  misc_feature (43)..(43): Xaa = His or Gln
  misc_feature (67)..(67): Xaa = Lys or Arg
  misc_feature (71)..(71): Xaa = Ile or Thr
  misc_feature (76)..(76): Xaa = Ile or Thr
  misc_feature (77)..(77): Xaa = Asn or Ser
  misc_feature (80)..(80): Xaa = Ser or Tyr
  misc_feature (83)..(83): Xaa = Leu or Val
  misc_feature (85)..(85): Xaa = Arg or Ser
  misc_feature (87)..(87): Xaa = Arg or Thr
  misc_feature (89)..(89): Xaa = Asp or Glu
  misc_feature (91)..(91): Xaa = Ser or Thr
  misc_feature (112)..(112): Xaa = Ala or Gln
QVQLXQSGAEXXXPGASVKXSCKAXGFTFIDYEMHWVRQXPXXGLEWIGGIHPGSGGTAYNQKFKGXATLXADISXXTAXMEXSXLXSXDXAVYYCTREGFDVGWYFDVWGXGTTVTVSS

SEQ ID NO: 67 - protein, 107 aa, Artificial Sequence
  41D2-2C3D7 VL; 1910D2HzL4 VL
  misc_feature (3)..(3): Xaa = Gln or Val
  misc_feature (4)..(4): Xaa = Leu or Met
  misc_feature (8)..(8): Xaa = His or Pro
  misc_feature (9)..(9): Xaa = Lys or Ser
  misc_feature (11)..(11): Xaa = Leu or Met
  misc_feature (13)..(13): Xaa = Ala or Thr
  misc_feature (20)..(20): Xaa = Ser or Thr
  misc_feature (42)..(42): Xaa = Lys or Gln
  misc_feature (43)..(43): Xaa = Ala or Ser
  misc_feature (60)..(60): Xaa = Asp or Ser
  misc_feature (63)..(63): Xaa = Ser or Thr
  misc_feature (70)..(70): Xaa = Asp or Glu
  misc_feature (77)..(77): Xaa = Asn or Ser
  misc_feature (78)..(78): Xaa = Leu or Val
  misc_feature (80)..(80): Xaa = Pro or Ser
  misc_feature (83)..(83): Xaa = Phe or Leu
  misc_feature (85)..(85): Xaa = Asp or Thr
  misc_feature (104)..(104): Xaa = Leu or Val
  misc_feature (106)..(106): Xaa = Ile or Val
DIXXTQSXXFXSXSVGDRVXITCKASQDVGTAVAWYQQKPGXXPKLLIYWASTRHTGVPXRFXGSGSGTXFTLTISXXQXEDXAXYFCQQYSSYPWTFGGGTKXEXK

SEQ ID NO: 68 - protein, 112 aa, Artificial Sequence
  46H3A8 VL; 1910h3hzL3 VL
  misc_feature (3)..(3): Xaa = Leu or Val
  misc_feature (7)..(7): Xaa = Ser or Thr
  misc_feature (14)..(14): Xaa = Ser or Thr
  misc_feature (17)..(17): Xaa = Asp or Gln
  misc_feature (18)..(18): Xaa = Pro or Gln
  misc_feature (42)..(42): Xaa = Leu or Gln
  misc_feature (44)..(44): Xaa = Lys or Arg
  misc_feature (50)..(50): Xaa = Lys or Arg
  misc_feature (85)..(85): Xaa = Ala or Gly
  misc_feature (88)..(88): Xaa = Leu or Val
  misc_feature (105)..(105): Xaa = Gly or Gln
DVXMTQXPLSLPVXLGXXASISCRSSQSIVHSDGDTFLEWYXQXPGQSPXLLIYKVSNRFSGVPDRFSGSGSGTDFTLKISRVEXEDXGVYYCFQGSHVPYTFGXGTKLEIK

SEQ ID NO: 69 - protein, 23 aa, Artificial Sequence
  41D2-2C3D7 L-FR1; 1910D2HzL4 L-FR1
  misc_feature (3)..(3): Xaa = Gln or Val
  misc_feature (4)..(4): Xaa = Leu or Met
  misc_feature (8)..(8): Xaa = His or Pro
  misc_feature (9)..(9): Xaa = Lys or Ser
  misc_feature (11)..(11): Xaa = Leu or Met
  misc_feature (13)..(13): Xaa = Ala or Thr
  misc_feature (20)..(20): Xaa = Ser or Thr
DIXXTQSXXFXSXSVGDRVXITC

SEQ ID NO: 70 - protein, 23 aa, Artificial Sequence
  46H3A8 L-FR1; 1910h3hzL3 L-FR1
  misc_feature (3)..(3): Xaa = Leu or Val
  misc_feature (7)..(7): Xaa = Ser or Thr
  misc_feature (14)..(14): Xaa = Ser or Thr
  misc_feature (17)..(17): Xaa = Asp or Gln
  misc_feature (18)..(18): Xaa = Pro or Gln
DVXMTQXPLSLPVXLGXXASISC

SEQ ID NO: 71 - protein, 15 aa, Artificial Sequence
  41D2-2C3D7 L-FR2; 1910D2HzL4 L-FR2
  misc_feature (8)..(8): Xaa = Lys or Gln
  misc_feature (9)..(9): Xaa = Ala or Ser
WYQQKPGXXPKLLIY

SEQ ID NO: 72 - protein, 15 aa, Artificial Sequence
  46H3A8 L-FR2; 1910h3hzL3 L-FR2
  misc_feature (3)..(3): Xaa = Leu or Gln
  misc_feature (5)..(5): Xaa = Lys or Arg
  misc_feature (11)..(11): Xaa = Lys or Arg
WYXQXPGQSPXLLIY

SEQ ID NO: 73 - protein, 32 aa, Artificial Sequence
  41D2-2C3D7 L-FR3; 1910D2HzL4 L-FR3
  misc_feature (4)..(4): Xaa = Asp or Ser
  misc_feature (7)..(7): Xaa = Ser or Thr
  misc_feature (14)..(14): Xaa = Asp or Glu
  misc_feature (21)..(21): Xaa = Asn or Ser
  misc_feature (22)..(22): Xaa = Leu or Val
  misc_feature (24)..(24): Xaa = Pro or Ser
  misc_feature (27)..(27): Xaa = Phe or Leu
  misc_feature (29)..(29): Xaa = Asp or Thr
GVPXRFXGSGSGTXFTLTISXXQXEDXAXYFC

SEQ ID NO: 74 - protein, 32 aa, Artificial Sequence
  46H3A8 L-FR3; 1910h3hzL3 L-FR3
  misc_feature (24)..(24): Xaa = Ala or Gly
  misc_feature (27)..(27): Xaa = Leu or Val
GVPDRFSGSGSGTDFTLKISRVEXEDXGVYYC

SEQ ID NO: 75 - protein, 10 aa, Artificial Sequence
  41D2-2C3D7 L-FR4; 1910D2HzL4 L-FR4
  misc_feature (7)..(7): Xaa = Leu or Val
  misc_feature (9)..(9): Xaa = Ile or Val
FGGGTKXEXK

SEQ ID NO: 76 - protein, 10 aa, Artificial Sequence
  46H3A8 L-FR4; 1910h3hzL3 L-FR4
  misc_feature (3)..(3): Xaa = Gly or Gln
FGXGTKLEIK

SEQ ID NO: 77 - protein, 327 aa, Artificial Sequence
  1910h3hzH4 heavy chain constant region
ASTKGPSVFPLAPCSRSTSESTAALGCLVKDYFPEPVTVSWNSGALTSGVHTFPAVLQSSGLYSLSSVVTVPSSSLGTKTYTCNVDHKPSNTKVDKRVESKYGPPCPPCPAPEFLGGPSVFLFPPKPKDTLMISRTPEVTCVVVDVSQEDPEVQFNWYVDGVEVHNAKTKPREEQFNSTYRVVSVLTVLHQDWLNGKEYKCKVSNKGLPSSIEKTISKAKGQPREPQVYTLPPSQEEMTKNQVSLTCLVKGFYPSDIAVEWESNGQPENNYKTTPPVLDSDGSFFLYSRLTVDKSRWQEGNVFSCSVMHEALHNHYTQKSLSLSLGK

SEQ ID NO: 78 - protein, 107 aa, Artificial Sequence [sequence omitted]

SEQ ID NO: 79 - protein, 447 aa, Artificial Sequence
  1910h3hzH4 heavy chain
QVQLVQSGAEVKKPGASVKVSCKASGFTFIDYEMHWVRQAPGQGLEWIGGIHPGSGGTAYNQKFKGRATLTADISISTAYMELSRLRSDDTAVYYCTREGFDVGWYFDVWGQGTTVTVSSASTKGPSVFPLAPCSRSTSESTAALGCLVKDYFPEPVTVSWNSGALTSGVHTFPAVLQSSGLYSLSSVVTVPSSSLGTKTYTCNVDHKPSNTKVDKRVESKYGPPCPPCPAPEFLGGPSVFLFPPKPKDTLMISRTPEVTCVVVDVSQEDPEVQFNWYVDGVEVHNAKTKPREEQFNSTYRVVSVLTVLHQDWLNGKEYKCKVSNKGLPSSIEKTISKAKGQPREPQVYTLPPSQEEMTKNQVSLTCLVKGFYPSDIAVEWESNGQPENNYKTTPPVLDSDGSFFLYSRLTVDKSRWQEGNVFSCSVMHEALHNHYTQKSLSLSLGK

SEQ ID NO: 80 - protein, 219 aa, Artificial Sequence
  1910h3hzL3 light chain
DVVMTQSPLSLPVTLGQPASISCRSSQSIVHSDGDTFLEWYQQRPGQSPRLLIYKVSNRFSGVPDRFSGSGSGTDFTLKISRVEAEDVGVYYCFQGSHVPYTFGQGTKLEIKRTVAAPSVFIFPPSDEQLKSGTASVVCLLNNFYPREAKVQWKVDNALQSGNSQESVTEQDSKDSTYSLSSTLTLSKADYEKHKVYACEVTHQGLSSPVTKSFNRGEC

SEQ ID NO: 81 - protein, 327 aa, Artificial Sequence; identical to SEQ ID NO: 77
  1910D2HzH3 heavy chain constant region

SEQ ID NO: 82 - protein, 107 aa, Artificial Sequence [sequence omitted]

SEQ ID NO: 83 - protein, 443 aa, Artificial Sequence
  1910D2HzH3 heavy chain
EVQLVESGGGLVKPGGSLRLSCAASGFTFSNYDMSWVRQAPGKGLEWVSTISGGGSYTYYADSVKGRFTISRDNAKNSLYLQMNSLRAEDTAVYYCVSPYYGMEYWGQGTLVTVSSASTKGPSVFPLAPCSRSTSESTAALGCLVKDYFPEPVTVSWNSGALTSGVHTFPAVLQSSGLYSLSSVVTVPSSSLGTKTYTCNVDHKPSNTKVDKRVESKYGPPCPPCPAPEFLGGPSVFLFPPKPKDTLMISRTPEVTCVVVDVSQEDPEVQFNWYVDGVEVHNAKTKPREEQFNSTYRVVSVLTVLHQDWLNGKEYKCKVSNKGLPSSIEKTISKAKGQPREPQVYTLPPSQEEMTKNQVSLTCLVKGFYPSDIAVEWESNGQPENNYKTTPPVLDSDGSFFLYSRLTVDKSRWQEGNVFSCSVMHEALHNHYTQKSLSLSLGK

SEQ ID NO: 84 - protein, 214 aa, Artificial Sequence
  1910D2HzL4 light chain
DIQLTQSPSFLSASVGDRVTITCKASQDVGTAVAWYQQKPGKAPKLLIYWASTRHTGVPSRFSGSGSGTEFTLTISSLQPEDFATYFCQQYSSYPWTFGGGTKVEIKRTVAAPSVFIFPPSDEQLKSGTASVVCLLNNFYPREAKVQWKVDNALQSGNSQESVTEQDSKDSTYSLSSTLTLSKADYEKHKVYACEVTHQGLSSPVTKSFNRGEC

SEQ ID NO: 85 - protein, 6 aa, Artificial Sequence
  Ab2005Am08 HCDR2
SGGGRY

SEQ ID NO: 86 - protein, 116 aa, Artificial Sequence
  Ab2005Am08 VH
EVQLVESGGGLVKPGGSLRLSCAASGFTFSNYDMSWVRQAPGKGLEWVSTISGGGRYTYYADSVKGRFTISRDNAKNSLYLQMNSLRAEDTAVYYCVSPYYGMEYWGQGTLVTVSS

SEQ ID NO: 87 - protein, 446 aa, Artificial Sequence
  Ab2005Am08 heavy chain
EVQLVESGGGLVKPGGSLRLSCAASGFTFSNYDMSWVRQAPGKGLEWVSTISGGGRYTYYADSVKGRFTISRDNAKNSLYLQMNSLRAEDTAVYYCVSPYYGMEYWGQGTLVTVSSASTKGPSVFPLAPSSKSTSGGTAALGCLVKDYFPEPVTVSWNSGALTSGVHTFPAVLQSSGLYSLSSVVTVPSSSLGTQTYICNVNHKPSNTKVDKKVEPKSCDKTHTCPPCPAPEAAGGPSVFLFPPKPKDTLMISRTPEVTCVVVSVSHEDPEVKFNWYVDGVEVHNAKTKPREEQYNSTYRVVSVLTVLHQDWLNGKEYKCKVSNKALPAPIEKTISKAKGQPREPQVYTLPPSREEMTKNQVSLTCLVKGFYPSDIAVEWESNGQPENNYKTTPPVLDSDGSFFLYSKLTVDKSRWQQGNVFSCSVMHEALHNHYTQKSLSLSPGK